European Patent Specification EP 3 980 786 B1, published October 16, 2024. Title: METHODS OF IDENTIFYING CRITICAL QUALITY ATRIBUTES. Applicant: Amgen Inc. The sequence listing filed with the application follows.

SEQUENCE LISTING (88 sequences)

SEQ ID NO: 1 - skipped

SEQ ID NO: 2 - protein, 470 aa, Homo sapiens [sequence omitted]

SEQ ID NO: 3 - protein, 235 aa, Homo sapiens
METPAQLLFLLLLWLPDTTGEIVLTQSPGTLSLSPGDRATLSCRASQSVSSSYFAWYQQKPGQAPRLLIYGASSRATGIPDRFSGSGSGTDFTLTISRLEPEDFAVYYCQQYDRSPRTFGQGTKVEIKRTVAAPSVFIFPPSDEQLKSGTASVVCLLNNFYPREAKVQWKVDNALQSGNSQESVTEQDSKDSTYSLSSTLTLSKADYEKHKVYACEVTHQGLSSPVTKSFNRGEC

SEQ ID NO: 4 - protein, 463 aa, Homo sapiens
MDWTWRILFLVAAATGAHSQVQLVQSGAEVKKPGASVKVSCKSSGYTFTGYYMHWVRQAPGQGLEWMGWINPNSGGTNYAQKFKGRVTMTRDTSISTAYMELSRLRSDDTAVYYCARDKWLDGFDYWGQGTLVTVSSASTKGPSVFPLAPCSRSTSESTAALGCLVKDYFPEPVTVSWNSGALTSGVHTFPAVLQSSGLYSLSSVVTVPSSNFGTQTYTCNVDHKPSNTKVDKTVERKCCVECPPCPAPPVAGPSVFLFPPKPKDTLMISRTPEVTCVVVDVSHEDPEVQFNWYVDGVEVHNAKTKPREEQFNSTFRVVSVLTVVHQDWLNGKEYKCKVSNKGLPAPIEKTISKTKGQPREPQVYTLPPSREEMTKNQVSLTCLVKGFYPSDIAVEWESNGQPENNYKTTPPMLDSDGSFFLYSKLTVDKSRWQQGNVFSCSVMHEALHNHYTQKSLSLSPGK

SEQ ID NO: 5 - protein, 235 aa, Homo sapiens
MAWALLLLTLLTQDTGSWAQSVLTQSPSASGTPGQRVTISCSGSSSNIGSNYVYWYQQLPGAAPKLLILRNNQRPSGVPDRFSGSKSGTSASLTISGLRSEDEADYYCAAWDDSLSGWVFGGGTKLTVLGQPKANPTVTLFPPSSEELQANKATLVCLISDFYPGAVTVAWKADGSPVKAGVETTKPSKQSNNKYAASSYLSLTPEQWKSHRSYSCQVTHEGSTVEKTVAPTECS

SEQ ID NO: 6 - protein, 479 aa, Homo sapiens
MDMRVPAQLLGLLLLWLRGARCEVQLVESGGGLVKPGGSLRLSCAASGFTFSNAWMSWVRQAPGKGLEWVGRIKSKTDGGTTDYTAPVKGRFTISRDDSKNTLYLQMNSLKAEDTAVYYCTTDRTGYSISWSSYYYYYGMDVWGQGTTVTVSSASTKGPSVFPLAPCSRSTSESTAALGCLVKDYFPEPVTVSWNSGALTSGVHTFPAVLQSSGLYSLSSVVTVPSSNFGTQTYTCNVDHKPSNTKVDKTVERKCCVECPPCPAPPVAGPSVFLFPPKPKDTLMISRTPEVTCVVVDVSHEDPEVQFNWYVDGVEVHNAKTKPREEQFNSTFRVVSVLTVVHQDWLNGKEYKCKVSNKGLPAPIEKTISKTKGQPREPQVYTLPPSREEMTKNQVSLTCLVKGFYPSDIAVEWESNGQPENNYKTTPPMLDSDGSFFLYSKLTVDKSRWQQGNVFSCSVMHEALHNHYTQKSLSLSPGK

SEQ ID NO: 7 - protein, 235 aa, Homo sapiens
METPAQLLFLLLLWLPDTTGEIVLTQSPGTLSLSPGERATLSCRASQSVRGRYLAWYQQKPGQAPRLLIYGASSRATGIPDRFSGSGSGTDFTLTISRLEPEDFAVFYCQQYGSSPRTFGQGTKVEIKRTVAAPSVFIFPPSDEQLKSGTASVVCLLNNFYPREAKVQWKVDNALQSGNSQESVTEQDSKDSTYSLSSTLTLSKADYEKHKVYACEVTHQGLSSPVTKSFNRGEC

SEQ ID NO: 8 - protein, 467 aa, Homo sapiens
MEFGLSWLFLVAILKGVQCEVQLLESGGGLVQPGGSLRLSCAASGFTFSSYAMSWVRQAPGKGLEWVSGITGSGGSTYYADSVKGRFTISRDNSKNTLYLQMNSLRAEDTAVYYCAKDPGTTVIMSWFDPWGQGTLVTVSSASTKGPSVFPLAPCSRSTSESTAALGCLVKDYFPEPVTVSWNSGALTSGVHTFPAVLQSSGLYSLSSVVTVPSSNFGTQTYTCNVDHKPSNTKVDKTVERKCCVECPPCPAPPVAGPSVFLFPPKPKDTLMISRTPEVTCVVVDVSHEDPEVQFNWYVDGVEVHNAKTKPREEQFNSTFRVVSVLTVVHQDWLNGKEYKCKVSNKGLPAPIEKTISKTKGQPREPQVYTLPPSREEMTKNQVSLTCLVKGFYPSDIAVEWESNGQPENNYKTTPPMLDSDGSFFLYSKLTVDKSRWQQGNVFSCSVMHEALHNHYTQKSLSLSPGK

SEQ ID NO: 9 - protein, 242 aa, Homo sapiens
MDMRVPAQLLGLLLLWLRGARCDIVMTQTPLSLPVTPGEPASISCRSSQSLLNSVDGSTNLDWYLQKPGQSPQLLIYTLSYRASGVPDRFSGSGSGTDFTLKISRVEAEDVGVYYCMQRIEFPLTFGGGTKVEIKRTVAAPSVFIFPPSDEQLKSGTASVVCLLNNFYPREAKVQWKVDNALQSGNSQESVTEQDSKDSTYSLSSTLTLSKADYEKHKVYACEVTHQGLSSPVTKSFNRGEC

SEQ ID NO: 10 - protein, 465 aa, Homo sapiens
MELGLCWVFLVAILEGVQCEVQLVESGGGLVQPGGSLRLSCAASGFTFSSYSMNWVRQAPGKGLEWVSYISSSGSSIYYADSVKGRFTISRDNAKNSLYLQMNSLRDEDTAVYYCARERYYGDTPFDYWGQGTLVTVSSASTKGPSVFPLAPCSRSTSESTAALGCLVKDYFPEPVTVSWNSGALTSGVHTFPAVLQSSGLYSLSSVVTVPSSNFGTQTYTCNVDHKPSNTKVDKTVERKCCVECPPCPAPPVAGPSVFLFPPKPKDTLMISRTPEVTCVVVDVSHEDPEVQFNWYVDGVEVHNAKTKPREEQFNSTFRVVSVLTVVHQDWLNGKEYKCKVSNKGLPAPIEKTISKTKGQPREPQVYTLPPSREEMTKNQVSLTCLVKGFYPSDIAVEWESNGQPENNYKTTPPMLDSDGSFFLYSKLTVDKSRWQQGNVFSCSVMHEALHNHYTQKSLSLSPGK

SEQ ID NO: 11 - protein, 233 aa, Homo sapiens
MSPSQLIGFLLLWVPASRGEIVLTQSPDFQSVTPKEKVTITCRASQSIGSSLHWYQQKPDQSPKLLIKYASQSFSGVPSRFSGSGSGTDFTLTINSLEAEDAAAYYCHQSSSLPLTFGGGTKVEIKRTVAAPSVFIFPPSDEQLKSGTASVVCLLNNFYPREAKVQWKVDNALQSGNSQESVTEQDSKDSTYSLSSTLTLSKADYEKHKVYACEVTHQGLSSPVTKSFNRGEC

SEQ ID NO: 12 - protein, 463 aa, Homo sapiens
MGSTAILALLLAVLQGVCAEVQLMQSGAEVKKPGESLKISCKGSGYSFSFHWIAWVRQMPGKGLEWMGIIHPGASDTRYSPSFQGQVTISADNSNSATYLQWSSLKASDTAMYFCARQRELDYFDYWGQGTLVTVSSASTKGPSVFPLAPCSRSTSESTAALGCLVKDYFPEPVTVSWNSGALTSGVHTFPAVLQSSGLYSLSSVVTVPSSNFGTQTYTCNVDHKPSNTKVDKTVERKCCVECPPCPAPPVAGPSVFLFPPKPKDTLMISRTPEVTCVVVDVSHEDPEVQFNWYVDGVEVHNAKTKPREEQFNSTFRVVSVLTVVHQDWLNGKEYKCKVSNKGLPAPIEKTISKTKGQPREPQVYTLPPSREEMTKNQVSLTCLVKGFYPSDIAVEWESNGQPENNYKTTPPMLDSDGSFFLYSKLTVDKSRWQQGNVFSCSVMHEALHNHYTQKSLSLSPGK

SEQ ID NO: 13 - protein, 236 aa, Homo sapiens
MDMRVPAQLLGLLLLWLRGARCDIQMTQSPSSLSASVGDRVTITCKASQDINKYVAWYQQKPGKAPKLLIYYTSWLQPGVPSRFSGSGSGTDFTFTISSLQPEDIATYYCLQYDNLLYTFGQGTKLEIKRTVAAPSVFIFPPSDEQLKSGTASVVCLLNNFYPREAKVQWKVDNALQSGNSQESVTEQDSKDSTYSLSSTLTLSKADYEKHKVYACEVTHQGLSSPVTKSFNRGEC

SEQ ID NO: 14 - protein, 467 aa, Homo sapiens
MDMRVPAQLLGLLLLWLRGARCEVQLVESGGGLVQPGGSLRLSCAASGFTFSRYWMNWVRQAPGKGLEWVAQIRLKSDNYATHYAESVKGRFTISRDNAKNSLYLQMNSLRAEDTAVYYCTEGLDYWGQGTTVTVSSASTKGPSVFPLAPSSKSTSGGTAALGCLVKDYFPEPVTVSWNSGALTSGVHTFPAVLQSSGLYSLSSVVTVPSSSLGTQTYICNVNHKPSNTKVDKKVEPKSCDKTHTCPPCPAPELLGGPSVFLFPPKPKDTLMISRTPEVTCVVVDVSHEDPEVKFNWYVDGVEVHNAKTKPREEQYNSTYRVVSVLTVLHQDWLNGKEYKCKVSNKALPAPIEKTISKAKGQPREPQVYTLPPSREEMTKNQVSLTCLVKGFYPSDIAVEWESNGQPENNYKTTPPVLDSDGSFFLYSKLTVDKSRWQQGNVFSCSVMHEALHNHYTQKSLSLSPGK

SEQ ID NO: 15 - protein, 236 aa, Homo sapiens
MDMRVLAQLLGLLLLCFPGARCDIQMTQSPSSLSASVGDRVTITCRASQGISNWLAWYQQKPEKAPKSLIYAASSLQSGVPSRFSGSGSGTDFTLTISSLQPEDFATYYCQQYDSYPRTFGQGTKVEIKRTVAAPSVFIFPPSDEQLKSGTASVVCLLNNFYPREAKVQWKVDNALQSGNSQESVTEQDSKDSTYSLSSTLTLSKADYEKHKVYACEVTHQGLSSPVTKSFNRGEC

SEQ ID NO: 16 - protein, 466 aa, Homo sapiens
MELGLNWVFLVAILEGVHCEVQLVESGGGLVQPGGSLRLSCAASGFTFSSYWMSWVRQAPGKGLEWVAYIKQDGNEKYYVDSVKGRFTISRDNAKNSLYLQMNSLRAEDTAVYYCAREGILWFGDLPTFWGQGTLVTVSSASTKGPSVFPLAPCSRSTSESTAALGCLVKDYFPEPVTVSWNSGALTSGVHTFPAVLQSSGLYSLSSVVTVPSSNFGTQTYTCNVDHKPSNTKVDKTVERKCCVECPPCPAPPVAGPSVFLFPPKPKDTLMISRTPEVTCVVVDVSHEDPEVQFNWYVDGVEVHNAKTKPREEQFNSTFRVVSVLTVVHQDWLNGKEYKCKVSNKGLPAPIEKTISKTKGQPREPQVYTLPPSREEMTKNQVSLTCLVKGFYPSDIAVEWESNGQPENNYKTTPPMLDSDGSFFLYSKLTVDKSRWQQGNVFSCSVMHEALHNHYTQKSLSLSPGK

SEQ ID NO: 17 - protein, 241 aa, Homo sapiens
MDMRLPAQLLGLLMLWVPGSSGDVLMTQSPLSLPVTLGQPASISCRSSQSIVHSNGNTYLEWYLQRPGQSPKLLIYKVSNRFSGVPDRFSGSGSGTDFTLKISRVEAEDVGVYYCFQGSHVPLTFGAGTKLEIKRTVAAPSVFIFPPSDEQLKSGTASVVCLLNNFYPREAKVQWKVDNALQSGNSQESVTEQDSKDSTYSLSSTLTLSKADYEKHKVYACEVTHQGLSSPVTKSFNRGEC

SEQ ID NO: 18 - protein, 470 aa, Homo sapiens
MDTLCSTLLLLTIPSWVLSQVTLKESGPALVKPTQTLTLTCTFSGFSLRTSGMGVGWIRQPPGKALEWLAHIWWDDDKSYNPSLKSQLTISKDTSKNQVVLTMTNMDPVDTATYYCARRNYYYDDYFAYWGQGTLVTVSSASTKGPSVFPLAPSSKSTSGGTAALGCLVKDYFPEPVTVSWNSGALTSGVHTFPAVLQSSGLYSLSSVVTVPSSSLGTQTYICNVNHKPSNTKVDKKVEPKSCDKTHTCPPCPAPELLGGPSVFLFPPKPKDTLMISRTPEVTCVVVDVSHEDPEVKFNWYVDGVEVHNAKTKPREEQYNSTYRVVSVLTVLHQDWLNGKEYKCKVSNKALPAPIEKTISKAKGQPREPQVYTLPPSRDELTKNQVSLTCLVKGFYPSDIAVEWESNGQPENNYKTTPPVLDSDGSFFLYSKLTVDKSRWQQGNVFSCSVMHEALHNHYTQKSLSLSPGK

SEQ ID NO: 19 - protein, 235 aa, Homo sapiens
METPAQLLFLLLLWLPDTTGEIVLTQSPGTLSLSPGERATLSCRASQSVSSSYFAWYQQKPGQAPRLLIYGTSSRATGIPDRFSGSGSGTDFTLTVSRLEPEDFAVYYCQQYDRSPRTFGQGTKVEIKRTVAAPSVFIFPPSDEQLKSGTASVVCLLNNFYPREAKVQWKVDNALQSGNSQESVTEQDSKDSTYSLSSTLTLSKADYEKHKVYACEVTHQGLSSPVTKSFNRGEC

SEQ ID NO: 20 - protein, 463 aa, Homo sapiens
MDWTWRILFLVAAATGAHSQVQLVQSGAAVKKPGASVKVSCKASGYTFTGYYIHWVRQAPGQGLEWMGWINPNSGGTNYAQKFQGRVTMTRDTSISTASMELSRLRSDDTAVYFCARDRWLDAFDIWGQGTMVTVSSASTKGPSVFPLAPCSRSTSESTAALGCLVKDYFPEPVTVSWNSGALTSGVHTFPAVLQSSGLYSLSSVVTVPSSNFGTQTYTCNVDHKPSNTKVDKTVERKCCVECPPCPAPPVAGPSVFLFPPKPKDTLMISRTPEVTCVVVDVSHEDPEVQFNWYVDGVEVHNAKTKPREEQFNSTFRVVSVLTVVHQDWLNGKEYKCKVSNKGLPAPIEKTISKTKGQPREPQVYTLPPSREEMTKNQVSLTCLVKGFYPSDIAVEWESNGQPENNYKTTPPMLDSDGSFFLYSKLTVDKSRWQQGNVFSCSVMHEALHNHYTQKSLSLSPGK

SEQ ID NO: 21 - protein, 235 aa, Homo sapiens
METPAQLLFLLLLWLPDTTGEIVLTQSPGTLSLSPGERATLSCRASQSVSSGYLTWYQQKPGQAPRLLIYGASSRATGIPDRFSGSGSGTDFTLTISRLEPEDFAVYYCQQYGNSLSRFGQGTKLEIKRTVAAPSVFIFPPSDEQLKSGTASVVCLLNNFYPREAKVQWKVDNALQSGNSQESVTEQDSKDSTYSLSSTLTLSKADYEKHKVYACEVTHQGLSSPVTKSFNRGEC

SEQ ID NO: 22 - protein, 474 aa, Homo sapiens
MDMRVPAQLLGLLLLWLRGARCQVQLVESGGGVVQPGRSLRLSCAASGFTFSSYGMHWVRQAPGKGLEWVAVIWYDGSNKYYADSVKGRFIISRDKSKNTLYLQMNSLRAEDTAVYYCARAGGIAAAGLYYYYGMDVWGQGTTVTVSSASTKGPSVFPLAPCSRSTSESTAALGCLVKDYFPEPVTVSWNSGALTSGVHTFPAVLQSSGLYSLSSVVTVPSSNFGTQTYTCNVDHKPSNTKVDKTVERKCCVECPPCPAPPVAGPSVFLFPPKPKDTLMISRTPEVTCVVVDVSHEDPEVQFNWYVDGVEVHNAKTKPREEQFNSTFRVVSVLTVVHQDWLNGKEYKCKVSNKGLPAPIEKTISKTKGQPREPQVYTLPPSREEMTKNQVSLTCLVKGFYPSDIAVEWESNGQPENNYKTTPPMLDSDGSFFLYSKLTVDKSRWQQGNVFSCSVMHEALHNHYTQKSLSLSPGK

SEQ ID NO: 23 - protein, 236 aa, Homo sapiens
MDMRVPAQLLGLLLLWLRGARCSSELTQDPTVSVALGQTVKITCQGDSLRSFYASWYQQKPGQAPVLVFYGKNNRPSGIPDRFSGSSSGNTASLTITGAQAEDEADYYCNSRDSSVYHLVLGGGTKLTVLGQPKANPTVTLFPPSSEELQANKATLVCLISDFYPGAVTVAWKADGSPVKAGVETTKPSKQSNNKYAASSYLSLTPEQWKSHRSYSCQVTHEGSTVEKTVAPTECS

SEQ ID NO: 24 - protein, 478 aa, Homo sapiens
MDMRVPAQLLGLLLLWLRGARCQVQLVQSGAEVKKPGASVKVSCKASGYTFTGYYMHWVRQAPGQGLEWMGWINPNSGGTNYAQKFQGRVTMTRDTSISTAYMELSRLRSDDTAVYFCARDQMSIIMLRGVFPPYYYGMDVWGQGTTVTVSSASTKGPSVFPLAPCSRSTSESTAALGCLVKDYFPEPVTVSWNSGALTSGVHTFPAVLQSSGLYSLSSVVTVPSSNFGTQTYTCNVDHKPSNTKVDKTVERKCCVECPPCPAPPVAGPSVFLFPPKPKDTLMISRTPEVTCVVVDVSHEDPEVQFNWYVDGVEVHNAKTKPREEQFNSTFRVVSVLTVVHQDWLNGKEYKCKVSNKGLPAPIEKTISKTKGQPREPQVYTLPPSREEMTKNQVSLTCLVKGFYPSDIAVEWESNGQPENNYKTTPPMLDSDGSFFLYSKLTVDKSRWQQGNVFSCSVMHEALHNHYTQKSLSLSPGK

SEQ ID NO: 25 - protein, 241 aa, Homo sapiens
MDMRVPAQLLGLLLLWLRGARCDIVMTQSPLSLPVTPGEPASISCRSSQSLLHSNGYNYLDWYLQKPGQSPQLLIYLGSNRASGVPDRFSGSGSGTDFTLKISRVEAEDVGVYYCMQALQTPLTFGGGTKVEIKRTVAAPSVFIFPPSDEQLKSGTASVVCLLNNFYPREAKVQWKVDNALQSGNSQESVTEQDSKDSTYSLSSTLTLSKADYEKHKVYACEVTHQGLSSPVTKSFNRGEC

SEQ ID NO: 26 - protein, 475 aa, Homo sapiens
MDMRVPAQLLGLLLLWLRGARCEVQLVESGGGLVQPGGSLRLSCAASGFTFSSYWMSWVRQAPGKGLEWVASIKQDGSEKYYVDSVKGRFTISRDNARNSLYLQMNSLRAEDTAVYYCARDLVLMVYDIDYYYYGMDVWGQGTTVTVSSASTKGPSVFPLAPCSRSTSESTAALGCLVKDYFPEPVTVSWNSGALTSGVHTFPAVLQSSGLYSLSSVVTVPSSNFGTQTYTCNVDHKPSNTKVDKTVERKCCVECPPCPAPPVAGPSVFLFPPKPKDTLMISRTPEVTCVVVDVSHEDPEVQFNWYVDGVEVHNAKTKPREEQFNSTFRVVSVLTVVHQDWLNGKEYKCKVSNKGLPAPIEKTISKTKGQPREPQVYTLPPSREEMTKNQVSLTCLVKGFYPSDIAVEWESNGQPENNYKTTPPMLDSDGSFFLYSKLTVDKSRWQQGNVFSCSVMHEALHNHYTQKSLSLSPGK

SEQ ID NO: 27 - protein, 241 aa, Homo sapiens
MDMRVPAQLLGLLLLWLRGARCDIVMTQSPLSLPVTPGEPASISCRSSQSLLHSNGYNYLDWYLQKPGQSPQLLIYLGSNRASGVPDRFSGSGSGTHLTLKISRVEAEDVGVYYCMQTLQTPLTFGGGTKVEIKRTVAAPSVFIFPPSDEQLKSGTASVVCLLNNFYPREAKVQWKVDNALQSGNSQESVTEQDSKDSTYSLSSTLTLSKADYEKHKVYACEVTHQGLSSPVTKSFNRGEC

SEQ ID NO: 28 - protein, 475 aa, Homo sapiens
MDMRVPAQLLGLLLLWLRGARCEVQLVESGGGLVQPGGSLRLSCAASGFTFSNYWMSWVRQAPGKGLEWVASIKQDGSEKYYVDSVKGRFAISRDNAKNSLFLQMNSLRAEDTAVYYCARDLVLMVYDIDYYYYGMDVWGQGTTVTVSSASTKGPSVFPLAPCSRSTSESTAALGCLVKDYFPEPVTVSWNSGALTSGVHTFPAVLQSSGLYSLSSVVTVPSSNFGTQTYTCNVDHKPSNTKVDKTVERKCCVECPPCPAPPVAGPSVFLFPPKPKDTLMISRTPEVTCVVVDVSHEDPEVQFNWYVDGVEVHNAKTKPREEQFNSTFRVVSVLTVVHQDWLNGKEYKCKVSNKGLPAPIEKTISKTKGQPREPQVYTLPPSREEMTKNQVSLTCLVKGFYPSDIAVEWESNGQPENNYKTTPPMLDSDGSFFLYSKLTVDKSRWQQGNVFSCSVMHEALHNHYTQKSLSLSPGK

SEQ ID NO: 29 - protein, 235 aa, Homo sapiens
MTCSPLLLTLLIHCTGSWAQSVLTQPPSVSAAPGQKVTISCSGSSSNIGNNYVSWYQQLPGTAPKLLIYDNNKRPSGIPDRFSGSKSGTSTTLGITGLQTGDEADYYCGTWDSRLSAVVFGGGTKLTVLGQPKANPTVTLFPPSSEELQANKATLVCLISDFYPGAVTVAWKADGSPVKAGVETTKPSKQSNNKYAASSYLSLTPEQWKSHRSYSCQVTHEGSTVEKTVAPTECS

SEQ ID NO: 30 - protein, 475 aa, Homo sapiens
MEFGLSWVFLVALLRGVQCQVQLVESGGGVVQPGRSLRLSCAASGFTFSSFGMHWVRQAPGKGLEWVAVISFDGSIKYSVDSVKGRFTISRDNSKNTLFLQMNSLRAEDTAVYYCARDRLNYYDSSGYYHYKYYGMAVWGQGTTVTVSSASTKGPSVFPLAPCSRSTSESTAALGCLVKDYFPEPVTVSWNSGALTSGVHTFPAVLQSSGLYSLSSVVTVPSSNFGTQTYTCNVDHKPSNTKVDKTVERKCCVECPPCPAPPVAGPSVFLFPPKPKDTLMISRTPEVTCVVVDVSHEDPEVQFNWYVDGVEVHNAKTKPREEQFNSTFRVVSVLTVVHQDWLNGKEYKCKVSNKGLPAPIEKTISKTKGQPREPQVYTLPPSREEMTKNQVSLTCLVKGFYPSDIAVEWESNGQPENNYKTTPPMLDSDGSFFLYSKLTVDKSRWQQGNVFSCSVMHEALHNHYTQKSLSLSPGK

SEQ ID NO: 31 - protein, 234 aa, Homo sapiens
MDMRVPAQLLGLLLLWLRGARCYELTQPPSVSVSPGQTATITCSGDKLGERYASWYQQRPGQSPVLVIYQDIKRPSGIPERFSGSNSGNTATLTISGTQAMDEADYFCQAWYSSTNVLFGGGTKLTVLGQPKAAPSVTLFPPSSEELQANKATLVCLISDFYPGAVTVAWKADSSPVKAGVETTTPSKQSNNKYAASSYLSLTPEQWKSHRSYSCQVTHEGSTVEKTVAPTECS

SEQ ID NO: 32 - protein, 466 aa, Homo sapiens
MEFGLSWVFLVALLRGVQCQVQLVESGGGVVQPGRSLRLSCAASGFTFSSYGMHWVRQAPGKGLEWVAVIWYAESNKYYADSVKGRFTISRDNSKNTLYLQMNSLRAEDTAVYYCARAQEGIAPDAFDIWGQGTMVTVSSASTKGPSVFPLAPCSRSTSESTAALGCLVKDYFPEPVTVSWNSGALTSGVHTFPAVLQSSGLYSLSSVVTVPSSNFGTQTYTCNVDHKPSNTKVDKTVERKCCVECPPCPAPPVAGPSVFLFPPKPKDTLMISRTPEVTCVVVDVSHEDPEVQFNWYVDGVEVHNAKTKPREEQFNSTFRVVSVLTVVHQDWLNGKEYKCKVSNKGLPAPIEKTISKTKGQPREPQVYTLPPSREEMTKNQVSLTCLVKGFYPSDIAVEWESNGQPENNYKTTPPMLDSDGSFFLYSKLTVDKSRWQQGNVFSCSVMHEALHNHYTQKSLSLSPGK

SEQ ID NO: 33 - protein, 234 aa, Homo sapiens
MGSTAILGLLLAVLQGGRAEIVLTQSPGTLSLSPGERATLSCRASQSVSSSYLAWHQQKPGQAPRLLIYGASSRATGIPDRFSGSGSGTDFTLTISRLEPEDFAVYYCQQYGSSPWTFGQGTKVEIKRTVAAPSVFIFPPSDEQLKSGTASVVCLLNNFYPREAKVQWKVDNALQSGNSQESVTEQDSKDSTYSLSSTLTLSKADYEKHKVYACEVTHQGLSSPVTKSFNRGEC

SEQ ID NO: 34 - protein, 463 aa, Homo sapiens
MGSTAILGLLLAVLQGGRAEVQLLESGGGLVQPGGSLRLSCAASGFTFSTYVMSWVRQAPGKGLEWVSSISGSGLGSYYADSVKGRFTISRDNSKNTLYLQMNSLRAEDTAVYYCAKEAHRGPFDYWGQGTLVTVSSASTKGPSVFPLAPCSRSTSESTAALGCLVKDYFPEPVTVSWNSGALTSGVHTFPAVLQSSGLYSLSSVVTVPSSNFGTQTYTCNVDHKPSNTKVDKTVERKCCVECPPCPAPPVAGPSVFLFPPKPKDTLMISRTPEVTCVVVDVSHEDPEVQFNWYVDGVEVHNAKTKPREEQFNSTFRVVSVLTVVHQDWLNGKEYKCKVSNKGLPAPIEKTISKTKGQPREPQVYTLPPSREEMTKNQVSLTCLVKGFYPSDIAVEWESNGQPENNYKTTPPMLDSDGSFFLYSKLTVDKSRWQQGNVFSCSVMHEALHNHYTQKSLSLSPGK

SEQ ID NO: 35 - protein, 239 aa, Homo sapiens
MRLLAQLLGLLMLWVPGSSGDIVMTQTPLSSPVTLGQPASISCRSSQSLVHSDGNTYLSWLQQRPGQPPRLLIYKKFNRFSGVPDRFSGSGAGTDFTLKISRVEAEDVGVYYCMQATQIPLTFGPGTKVDIKRTVAAPSVFIFPPSDEQLKSGTASVVCLLNNFYPREAKVQWKVDNALQSGNSQESVTEQDSKDSTYSLSSTLTLSKADYEKHKVYACEVTHQGLSSPVTKSFNRGEC

SEQ ID NO: 36 - protein, 472 aa, Homo sapiens
MEFGLSWVFLVALLRGVQCQVQLVESGGGVVQPGRSLRLSCAASGFTFSFYGMHWVRQAPGKGLEWVAVIWYDGSNKYYADSVKGRFTISRDNSKNTLYLQMNSLRAEDTAVYYCARGGYDYVWGSYRRNSDFDYWGQGTLVTVSSASTKGPSVFPLAPCSRSTSESTAALGCLVKDYFPEPVTVSWNSGALTSGVHTFPAVLQSSGLYSLSSVVTVPSSNFGTQTYTCNVDHKPSNTKVDKTVERKCCVECPPCPAPPVAGPSVFLFPPKPKDTLMISRTPEVTCVVVDVSHEDPEVQFNWYVDGVEVHNAKTKPREEQFNSTFRVVSVLTVVHQDWLNGKEYKCKVSNKGLPAPIEKTISKTKGQPREPQVYTLPPSREEMTKNQVSLTCLVKGFYPSDIAVEWESNGQPENNYKTTPPMLDSDGSFFLYSKLTVDKSRWQQGNVFSCSVMHEALHNHYTQKSLSLSPGK

SEQ ID NO: 37 - protein, 235 aa, Homo sapiens
MEAPAQLLFLLLLWLPDTTGEIVMTQSPATLSVSPGERATLSCRASQSVDSNLAWYRQKPGQAPRLLIYGASTRATGIPARFSGSGSGTEFTLTISSLQSEDFAVYYCQQYINWPPITFGQGTRLEIKRTVAAPSVFIFPPSDEQLKSGTASVVCLLNNFYPREAKVQWKVDNALQSGNSQESVTEQDSKDSTYSLSSTLTLSKADYEKHKVYACEVTHQGLSSPVTKSFNRGEC

SEQ ID NO: 38 - protein, 465 aa, Homo sapiens
MKHLWFFLLLVAAPRWVLSQVQLQESGPGLVKPSETLSLTCTVSGGSISIYYWSWIRQPPGKGLEWIGYVYYSGSTNYNPSLKSRVTISVDTSKNQFSLKLNSVTAADTAVYYCARGGYDFWSGYFDYWGQGTLVTVSSASTKGPSVFPLAPCSRSTSESTAALGCLVKDYFPEPVTVSWNSGALTSGVHTFPAVLQSSGLYSLSSVVTVPSSNFGTQTYTCNVDHKPSNTKVDKTVERKCCVECPPCPAPPVAGPSVFLFPPKPKDTLMISRTPEVTCVVVDVSHEDPEVQFNWYVDGVEVHNAKTKPREEQFNSTFRVVSVLTVVHQDWLNGKEYKCKVSNKGLPAPIEKTISKTKGQPREPQVYTLPPSREEMTKNQVSLTCLVKGFYPSDIAVEWESNGQPENNYKTTPPMLDSDGSFFLYSKLTVDKSRWQQGNVFSCSVMHEALHNHYTQKSLSLSPGK

SEQ ID NO: 39 - protein, 240 aa, Homo sapiens
MVLQTQVFISLLLWISGAYGDIVLTQSPDSLAVSLGERATINCKSSQSILYSSSNENFLTWYQQKPGQPPKLLIYWASTRESGVPDRFSGSGSGTDFTLTISSLQPEDVAVYYCQQYFSVFRTFGQGTRVEIKRTVAAPSVFIFPPSDEQLKSGTASVVCLLNNFYPREAKVQWKVDNALQSGNSQESVTEQDSKDSTYSLSSTLTLSKADYEKHKVYACEVTHQGLSSPVTKSFNRGEC

SEQ ID NO: 40 - protein, 465 aa, Homo sapiens
MDWTWRILFLVAAATGAHSQVQLVQSGAEVKKPGASVKVSCKASGYTFTGYYIHWVRQAPGQGLEWMGWINPNSGGTNSAQKFRGRVTMTRDTSISTAYMELSRLRSDDTAVYYCAREGGYSYGYFDYWGQGTLVTVSSASTKGPSVFPLAPCSRSTSESTAALGCLVKDYFPEPVTVSWNSGALTSGVHTFPAVLQSSGLYSLSSVVTVPSSNFGTQTYTCNVDHKPSNTKVDKTVERKCCVECPPCPAPPVAGPSVFLFPPKPKDTLMISRTPEVTCVVVDVSHEDPEVQFNWYVDGVEVHNAKTKPREEQFNSTFRVVSVLTVVHQDWLNGKEYKCKVSNKGLPAPIEKTISKTKGQPREPQVYTLPPSREEMTKNQVSLTCLVKGFYPSDIAVEWESNGQPENNYKTTPPMLDSDGSFFLYSKLTVDKSRWQQGNVFSCSVMHEALHNHYTQKSLSLSPGK

SEQ ID NO: 41 - protein, 236 aa, Homo sapiens
MDMRVPAQLLGLLLLWFPGARCDIQMTQSPSSLSASVGDRVTITCRASQGIRNDLGWYQQKPGKAPKRLIYAASSLQSGVPSRFSGSGSGTEFTLTISSVQPEDFVTYYCLQHNSNPLTFGGGTKVEIKRTVAAPSVFIFPPSDEQLKSGTASVVCLLNNFYPREAKVQWKVDNALQSGNSQESVTEQDSKDSTYSLSSTLTLSKADYEKHKVYACEVTHQGLSSPVTKSFNRGEC

SEQ ID NO: 42 - protein, 473 aa, Homo sapiens
MEFGLSWVFLVALLRGVQCQVQLVESGGGVVQPGRSLRLSCAASGFTFSSYGMHWVRQAPGKGLEWVAVMWYDGSNKDYVDSVKGRFTISRDNSKNTLYLQMNRLRAEDTAVYYCAREKDHYDILTGYNYYYGLDVWGQGTTVTVSSASTKGPSVFPLAPCSRSTSESTAALGCLVKDYFPEPVTVSWNSGALTSGVHTFPAVLQSSGLYSLSSVVTVPSSNFGTQTYTCNVDHKPSNTKVDKTVERKCCVECPPCPAPPVAGPSVFLFPPKPKDTLMISRTPEVTCVVVDVSHEDPEVQFNWYVDGVEVHNAKTKPREEQFNSTFRVVSVLTVVHQDWLNGKEYKCKVSNKGLPAPIEKTISKTKGQPREPQVYTLPPSREEMTKNQVSLTCLVKGFYPSDIAVEWESNGQPENNYKTTPPMLDSDGSFFLYSKLTVDKSRWQQGNVFSCSVMHEALHNHYTQKSLSLSPGK

SEQ ID NO: 43 - protein, 235 aa, Homo sapiens
METPAQLLFLLLLWLPDTTGEIVLTQSPGTLSLSPGERATLSCRASQYISNTYLAWFQQKPGQAPRLLIYGAATRATGIPDRFSGSGSGTDFTFTISRLEPEDFAVYYCQQYGSSPWTFGQGTTVEIKRTVAAPSVFIFPPSDEQLKSGTASVVCLLNNFYPREAKVQWKVDNALQSGNSQESVTEQDSKDSTYSLSSTLTLSKADYEKHKVYACEVTHQGLSSPVTKSFNRGEC

SEQ ID NO: 44 - protein, 463 aa, Homo sapiens
MDWTWRILFLVAAATGAHSQVQLVQSGAEVKKPGASVKVSCKASGYTFTGYYMHWVRQAPGQGLEWMGWINPNSGGTNYAQRFRGRVTMTRDTSISTAYMELSRLRSDDTAVYYCARAPYDWTFDYWGQGTLVTVSSASTKGPSVFPLAPCSRSTSESTAALGCLVKDYFPEPVTVSWNSGALTSGVHTFPAVLQSSGLYSLSSVVTVPSSNFGTQTYTCNVDHKPSNTKVDKTVERKCCVECPPCPAPPVAGPSVFLFPPKPKDTLMISRTPEVTCVVVDVSHEDPEVQFNWYVDGVEVHNAKTKPREEQFNSTFRVVSVLTVVHQDWLNGKEYKCKVSNKGLPAPIEKTISKTKGQPREPQVYTLPPSREEMTKNQVSLTCLVKGFYPSDIAVEWESNGQPENNYKTTPPMLDSDGSFFLYSKLTVDKSRWQQGNVFSCSVMHEALHNHYTQKSLSLSPGK

SEQ ID NO: 45 - protein, 236 aa, Homo sapiens
MDMRVPAQLLGLLLLWLRGARCDIQMTQSPSSVSASVGDRVTITCRASQGISNWLAWYQQKPGTAPKLLIYAASSLQSGVPSRFSGSGSGTDFTLTISSLQPEDFATYYCQQANSFPFTFGPGTKVDIKRTVAAPSVFIFPPSDEQLKSGTASVVCLLNNFYPREAKVQWKVDNALQSGNSQESVTEQDSKDSTYSLSSTLTLSKADYEKHKVYACEVTHQGLSSPVTKSFNRGEC

SEQ ID NO: 46 - protein, 469 aa, Homo sapiens
MDMRVPAQLLGLLLLWLRGARCQVQLVQSGTEVKKPGASMKVSCKASGYTFTSYYMHWVRQAPGQGLEWMGIINPSGDSTSYAQKFQGRVTMTRDTSTNTVYMELSSLRSEDTAMYYCARDVEVRGISHFDYWGQGTLVTVSSASTKGPSVFPLAPCSRSTSESTAALGCLVKDYFPEPVTVSWNSGALTSGVHTFPAVLQSSGLYSLSSVVTVPSSNFGTQTYTCNVDHKPSNTKVDKTVERKCCVECPPCPAPPVAGPSVFLFPPKPKDTLMISRTPEVTCVVVDVSHEDPEVQFNWYVDGVEVHNAKTKPREEQFNSTFRVVSVLTVVHQDWLNGKEYKCKVSNKGLPAPIEKTISKTKGQPREPQVYTLPPSREEMTKNQVSLTCLVKGFYPSDIAVEWESNGQPENNYKTTPPMLDSDGSFFLYSKLTVDKSRWQQGNVFSCSVMHEALHNHYTQKSLSLSPGK

SEQ ID NO: 47 - protein, 238 aa, Homo sapiens
MGWSCIILFLVATATGVHSDIQLTQSPSSLSASVGDRVTMSCKSSQSVLYSANHKNYLAWYQQKPGKAPKLLIYWASTRESGVPSRFSGSGSGTDFTFTISSLQPEDIATYYCHQYLSSWTFGGGTKVQIKRTVAAPSVFIFPPSDEQLKSGTASVVCLLNNFYPREAKVQWKVDNALQSGNSQESVTEQDSKDSTYSLSSTLTLSKADYEKHKVYACEVTHQGLSSPVTKSFNRGEC

SEQ ID NO: 48 - protein, 465 aa, Homo sapiens
MGWSCIILFLVATATGVHSQVQLVQSGAEVKKPGSSVKVSCKASGYTFTSYWLHWVRQAPGQGLEWIGYINPRNDYTEYNQNFKDKATITADESTNTAYMELSSLRSEDTAFYFCARRDITTFYWGQGTTVTVSSASTKGPSVFPLAPSSKSTSGGTAALGCLVKDYFPEPVTVSWNSGALTSGVHTFPAVLQSSGLYSLSSVVTVPSSSLGTQTYICNVNHKPSNTKVDKRVEPKSCDKTHTCPPCPAPELLGGPSVFLFPPKPKDTLMISRTPEVTCVVVDVSHEDPEVKFNWYVDGVEVHNAKTKPREEQYNSTYRVVSVLTVLHQDWLNGKEYKCKVSNKALPAPIEKTISKAKGQPREPQVYTLPPSREEMTKNQVSLTCLVKGFYPSDIAVEWESNGQPENNYKTTPPVLDSDGSFFLYSKLTVDKSRWQQGNVFSCSVMHEALHNHYTQKSLSLSPGK

SEQ ID NO: 49 - protein, 235 aa, Homo sapiens
METPAQLLFLLLLWLPDTTGEIVLTQSPGTLSLSPGERATLSCRASQSVSSSYLAWYQQKPGQAPRLLIYGASSRATGIPDRFSGSGSGTDFTLTISRLEPEDFAVYYCQRSGGSSFTFGPGTKVDIKRTVAAPSVFIFPPSDEQLKSGTASVVCLLNNFYPREAKVQWKVDNALQSGNSQESVTEQDSKDSTYSLSSTLTLSKADYEKHKVYACEVTHQGLSSPVTKSFNRGEC

SEQ ID NO: 50 - protein, 466 aa, Homo sapiens
MGSTAILALLLAVLQGVCAEVQLVQSGAEVKKPGESLKISCKGSGYNFTSYWIGWVRQMPGKGLELMGIIYPGDSDTRYSPSFQGQVTISADKSISTAYLQWSSLKASDTAMYYCGSGSYFYFDLWGRGTLVTVSSASTKGPSVFPLAPSSKSTSGGTAALGCLVKDYFPEPVTVSWNSGALTSGVHTFPAVLQSSGLYSLSSVVTVPSSSLGTQTYICNVNHKPSNTKVDKKVEPKSCDKTHTCPPCPAPELLGGPSVFLFPPKPKDTLMISRTPEVTCVVVDVSHEDPEVKFNWYVDGVEVHNAKTKPREEQYNSTYRVVSVLTVLHQDWLNGKEYKCKVSNKALPAPIEKTISKAKGQPREPQVYTLPPSRDELTKNQVSLTCLVKGFYPSDIAVEWESNGQPENNYKTTPPVLDSDGSFFLYSKLTVDKSRWQQGNVFSCSVMHEALHNHYTQKSLSLSPGK

SEQ ID NO: 51 - protein, 241 aa, Homo sapiens
MDMRVPAQLLGLLLLWLRGARCDIVMTQSPLSLPVTPGEPASISCRSSQSLLHSHGYNYLDWYLQKPGQSPQLLIYLGSNRASGVPDRFSGSGSGTDFTLKISRVEAEDVGVYYCMQGTHWPPTFGQGTKLEIKRTVAAPSVFIFPPSDEQLKSGTASVVCLLNNFYPREAKVQWKVDNALQSGNSQESVTEQDSKDSTYSLSSTLTLSKADYEKHKVYACEVTHQGLSSPVTKSFNRGEC

SEQ ID NO: 52 - protein, 470 aa, Homo sapiens
MDMRVPAQLLGLLLLWLRGARCEVQLVQSGGGVVQPGRSLRLSCAASGFTFSSYGMHWVRQAPGKGLEWVSYISSSGSTIYYADSVKGRFTISRDNAKNSLYLQMNSLRAEDTAVYYCARDLLDYDLLTGYGYWGQGTLVTVSSASTKGPSVFPLAPCSRSTSESTAALGCLVKDYFPEPVTVSWNSGALTSGVHTFPAVLQSSGLYSLSSVVTVPSSNFGTQTYTCNVDHKPSNTKVDKTVERKCCVECPPCPAPPVAGPSVFLFPPKPKDTLMISRTPEVTCVVVDVSHEDPEVQFNWYVDGVEVHNAKTKPREEQFNSTFRVVSVLTVVHQDWLNGKEYKCKVSNKGLPAPIEKTISKTKGQPREPQVYTLPPSREEMTKNQVSLTCLVKGFYPSDIAVEWESNGQPENNYKTTPPMLDSDGSFFLYSKLTVDKSRWQQGNVFSCSVMHEALHNHYTQKSLSLSPGK

SEQ ID NO: 53 - protein, 235 aa, Homo sapiens
METPAQLLFLLLLWLPDTTGEIVLTQSPGTLSLSPGERATLSCRASQGISRSYLAWYQQKPGQAPSLLIYGASSRATGIPDRFSGSGSGTDFTLTISRLEPEDFAVYYCQQFGSSPWTFGQGTKVEIKRTVAAPSVFIFPPSDEQLKSGTASVVCLLNNFYPREAKVQWKVDNALQSGNSQESVTEQDSKDSTYSLSSTLTLSKADYEKHKVYACEVTHQGLSSPVTKSFNRGEC

SEQ ID NO: 54 - protein, 471 aa, Homo sapiens
MKHLWFFLLLVAAPRWVLSQVQLQESGPGLVKPSQTLSLTCTVSGGSISSGDYFWSWIRQLPGKGLEWIGHIHNSGTTYYNPSLKSRVTISVDTSKKQFSLRLSSVTAADTAVYYCARDRGGDYYYGMDVWGQGTTVTVSSASTKGPSVFPLAPSSKSTSGGTAALGCLVKDYFPEPVTVSWNSGALTSGVHTFPAVLQSSGLYSLSSVVTVPSSSLGTQTYICNVNHKPSNTKVDKRVEPKSCDKTHTCPPCPAPELLGGPSVFLFPPKPKDTLMISRTPEVTCVVVDVSHEDPEVKFNWYVDGVEVHNAKTKPREEQYNSTYRVVSVLTVLHQDWLNGKEYKCKVSNKALPAPIEKTISKAKGQPREPQVYTLPPSREEMTKNQVSLTCLVKGFYPSDIAVEWESNGQPENNYKTTPPVLDSDGSFFLYSKLTVDKSRWQQGNVFSCSVMHEALHNHYTQKSLSLSPGK

SEQ ID NO: 55 - protein, 236 aa, Homo sapiens
MDMRVPAQLLGLLLLWLSGARCDIQMTQSPSSLSASVGDRVTITCQASQDISNYLNWYQQKPGKAPKLLIYDASNLETGVPSRFSGSGSGTDFTFTISSLQPEDIATYFCQHFDHLPLAFGGGTKVEIKRTVAAPSVFIFPPSDEQLKSGTASVVCLLNNFYPREAKVQWKVDNALQSGNSQESVTEQDSKDSTYSLSSTLTLSKADYEKHKVYACEVTHQGLSSPVTKSFNRGEC

SEQ ID NO: 56 - protein, 464 aa, Homo sapiens
MKHLWFFLLLVAAPRWVLSQVQLQESGPGLVKPSETLSLTCTVSGGSVSSGDYYWTWIRQSPGKGLEWIGHIYYSGNTNYNPSLKSRLTISIDTSKTQFSLKLSSVTAADTAIYYCVRDRVTGAFDIWGQGTMVTVSSASTKGPSVFPLAPCSRSTSESTAALGCLVKDYFPEPVTVSWNSGALTSGVHTFPAVLQSSGLYSLSSVVTVPSSNFGTQTYTCNVDHKPSNTKVDKTVERKCCVECPPCPAPPVAGPSVFLFPPKPKDTLMISRTPEVTCVVVDVSHEDPEVQFNWYVDGVEVHNAKTKPREEQFNSTFRVVSVLTVVHQDWLNGKEYKCKVSNKGLPAPIEKTISKTKGQPREPQVYTLPPSREEMTKNQVSLTCLVKGFYPSDIAVEWESNGQPENNYKTTPPMLDSDGSFFLYSKLTVDKSRWQQGNVFSCSVMHEALHNHYTQKSLSLSPGK

SEQ ID NO: 57 - protein, 236 aa, Homo sapiens
METPAQLLFLLLLWLPDTASEIVLTQSPGTLSLSPGERATLSCRASQSVSNSYLAWYQQKPGQAPRLLIYGASSRAPGIPDRFSGSGSGTDFTLTISRLEPEDFAVYYCQQYDHSAGWTFGQGTKVEIKRTVAAPSVFIFPPSDEQLKSGTASVVCLLNNFYPREAKVQWKVDNALQSGNSQESVTEQDSKDSTYSLSSTLTLSKADYEKHKVYACEVTHQGLSSPVTKSFNRGEC

SEQ ID NO: 58 - protein, 460 aa, Homo sapiens
MGSTAILGLLLAVLQGVASEVQLVESGGGLVQPGGSLRLSCAASGFTFSRNAMFWVRQAPGKGLEWVSGIGTGGATSYADSVKGRFTISRDNAKNSLYLQMNSLRAEDTAVYYCARGRYYFPWWGQGTLVTVSSASTKGPSVFPLAPCSRSTSESTAALGCLVKDYFPEPVTVSWNSGALTSGVHTFPAVLQSSGLYSLSSVVTVPSSNFGTQTYTCNVDHKPSNTKVDKTVERKCCVECPPCPAPPVAGPSVFLFPPKPKDTLMISRTPEVTCVVVDVSHEDPEVQFNWYVDGVEVHNAKTKPREEQFNSTFRVVSVLTVVHQDWLNGKEYKCKVSNKGLPAPIEKTISKTKGQPREPQVYTLPPSREEMTKNQVSLTCLVKGFYPSDIAVEWESNGQPENNYKTTPPMLDSDGSFFLYSKLTVDKSRWQQGNVFSCSVMHEALHNHYTQKSLSLSPGK

SEQ ID NO: 59 - protein, 234 aa, Homo sapiens
METPAQLLFLLLLWLPDTTGEIVLTQSPGTLSLSPGERATLSCRASQSVSSSYLAWYQQKPGQAPRLLIYGASRRATGIPDRFSGSGSGTDFTLTISRLEPEDFAVYYCQRYGSSHTFGQGTKLEISRTVAAPSVFIFPPSDEQLKSGTASVVCLLNNFYPREAKVQWKVDNALQSGNSQESVTEQDSKDSTYSLSSTLTLSKADYEKHKVYACEVTHQGLSSPVTKSFNRGEC

SEQ ID NO: 60 - protein, 467 aa, Homo sapiens
MGSTAILALLLAVLQGVCAEVQLVQSGAEVKKPGESLKISCKVSGYFFTTYWIGWVRQMPGKGLEYMGIIYPGDSDTRYSPSFQGQVTISADKSISTAYLQWSSLKASDTAMYYCARGGNWNCFDYWGQGTLVTVSSASTKGPSVFPLAPSSKSTSGGTAALGCLVKDYFPEPVTVSWNSGALTSGVHTFPAVLQSSGLYSLSSVVTVPSSSLGTQTYICNVNHKPSNTKVDKRVEPKSCDKTHTCPPCPAPELLGGPSVFLFPPKPKDTLMISRTPEVTCVVVDVSHEDPEVKFNWYVDGVEVHNAKTKPREEQYNSTYRVVSVLTVLHQDWLNGKEYKCKVSNKALPAPIEKTISKAKGQPREPQVYTLPPSRDELTKNQVSLTCLVKGFYPSDIAVEWESNGQPENNYKTTPPVLDSDGSFFLYSKLTVDKSRWQQGNVFSCSVMHEALHNHYTQKSLSLSPGK

SEQ ID NO: 61 - protein, 241 aa, Homo sapiens
MDMRVPAQLLGLLLLWLRGARCDVVMTQSPLSLPVTPGEPASISCRSSQSLLHSNGYNYLDWYLQKPGQSPQLLIYLGSNRASGVPDRFSGSGSGTDFTLKISRVEAEDVGVYYCMQGTHWPLTFGQGTKVEIKRTVAAPSVFIFPPSDEQLKSGTASVVCLLNNFYPREAKVQWKVDNALQSGNSQESVTEQDSKDSTYSLSSTLTLSKADYEKHKVYACEVTHQGLSSPVTKSFNRGEC

SEQ ID NO: 62 - protein, 471 aa, Homo sapiens
MDMRVPAQLLGLLLLWLRGARCQVQLQESGPGLVKPSGTLSLTCAVSGGSISSSNWWSWVRQPPGKGLEWIGEIYHSGSTNYNPSLKSRVTISVDKSKNQFSLKLSSVTAADTAVYYCARWTGRTDAFDIWGQGTMVTVSSASTKGPSVFPLAPSSKSTSGGTAALGCLVKDYFPEPVTVSWNSGALTSGVHTFPAVLQSSGLYSLSSVVTVPSSSLGTQTYICNVNHKPSNTKVDKKVEPKSCDKTHTCPPCPAPELLGGPSVFLFPPKPKDTLMISRTPEVTCVVVDVSHEDPEVKFNWYVDGVEVHNAKTKPREEQYNSTYRVVSVLTVLHQDWLNGKEYKCKVSNKALPAPIEKTISKAKGQPREPQVYTLPPSRDELTKNQVSLTCLVKGFYPSDIAVEWESNGQPENNYKTTPPVLDSDGSFFLYSKLTVDKSRWQQGNVFSCSVMHEALHNHYTQKSLSLSPGK

SEQ ID NO: 63 - protein, 234 aa, Homo sapiens
MEAPAQLLFLLLLWLPDTTGEIVMTQSPATLSVSPGERATLSCRASQSVSSNLAWFQQKPGQAPRPLIYDASTRATGVPARFSGSGSGTDFTLTISSLQSEDFAVYYCQQYDNWPLTFGGGTKVEIKRTVAAPSVFIFPPSDEQLKSGTASVVCLLNNFYPREAKVQWKVDNALQSGNSQESVTEQDSKDSTYSLSSTLTLSKADYEKHKVYACEVTHQGLSSPVTKSFNRGEC

SEQ ID NO: 64 - protein, 461 aa, Homo sapiens
MEWTWRVLFLVAAATGAHSQVQLVQSGAEVKKPGASVKVSCKASGYTFTRYGISWVRQAPGQGLEWMGWISTYSGNTNYAQKLQGRVTMTTDTSTSTAYMELRSLRSDDTAVYYCARRQLYFDYWGQGTLVTVSSASTKGPSVFPLAPCSRSTSESTAALGCLVKDYFPEPVTVSWNSGALTSGVHTFPAVLQSSGLYSLSSVVTVPSSNFGTQTYTCNVDHKPSNTKVDKTVERKCCVECPPCPAPPVAGPSVFLFPPKPKDTLMISRTPEVTCVVVDVSHEDPEVQFNWYVDGVEVHNAKTKPREEQFNSTFRVVSVLTVVHQDWLNGKEYKCKVSNKGLPAPIEKTISKTKGQPREPQVYTLPPSREEMTKNQVSLTCLVKGFYPSDIAVEWESNGQPENNYKTTPPMLDSDGSFFLYSKLTVDKSRWQQGNVFSCSVMHEALHNHYTQKSLSLSPGK

SEQ ID NO: 65 - protein, 239 aa, Homo sapiens
MRLPAQLLGLLMLWIPGSSADIVMTQTPLSLSVTPGQPASISCKSGQSLLHSDGKTYLYWYLQKPGQPPQFLIYEVSNRFSRVPDRFSGSGSGTDFTLRISRVEAEDVGIYYCMQSIQLPWTFGQGTQVEIKRTVAAPSVFIFPPSDEQLKSGTASVVCLLNNFYPREAKVQWKVDNALQSGNSQESVTEQDSKDSTYSLSSTLTLSKADYEKHKVYACEVTHQGLSSPVTKSFNRGEC

SEQ ID NO: 66 - protein, 459 aa, Homo sapiens
MEFGLSWVFLVALLRGVQCQVQLVESGGGVVQPGRSLRLSCAASGFTFSGYGMHWVRQAPGKGLEWVAVISYDGNDKYYADSVKGRFTISRDNAKNTLYLQMNSLRAEDTAVYYCARELRVLWGQGTLVTVSSASTKGPSVFPLAPCSRSTSESTAALGCLVKDYFPEPVTVSWNSGALTSGVHTFPAVLQSSGLYSLSSVVTVPSSNFGTQTYTCNVDHKPSNTKVDKTVERKCCVECPPCPAPPVAGPSVFLFPPKPKDTLMISRTPEVTCVVVDVSHEDPEVQFNWYVDGVEVHNAKTKPREEQFNSTFRVVSVLTVVHQDWLNGKEYKCKVSNKGLPAPIEKTISKTKGQPREPQVYTLPPSREEMTKNQVSLTCLVKGFYPSDIAVEWESNGQPENNYKTTPPMLDSDGSFFLYSKLTVDKSRWQQGNVFSCSVMHEALHNHYTQKSLSLSPGK

SEQ ID NO: 67 - protein, 235 aa, Homo sapiens
MDMRVPAQLLGLLLLWLRGARCDIQMTQSPSSLSASVGDRVTITCRASQDISSYLNWYQQKPGKAPKLLIYSTSRLNSGVPSRFSGSGSGTDFTLTISSLQPEDFATYYCQQDIKHPTFGQGTKVEIKRTVAAPSVFIFPPSDEQLKSGTASVVCLLNNFYPREAKVQWKVDNALQSGNSQESVTEQDSKDSTYSLSSTLTLSKADYEKHKVYACEVTHQGLSSPVTKSFNRGEC

SEQ ID NO: 68 - protein, 465 aa, Homo sapiens
MDWTWRILFLVAAATGAHSEVQLVQSGAEVKKPGSSVKVSCKASGFTFTDYIMHWVRQAPGQGLEWMGYINPYNDDTEYNEKFKGRVTITADKSTSTAYMELSSLRSEDTAVYYCARSIYYYDAPFAYWGQGTLVTVSSASTKGPSVFPLAPCSRSTSESTAALGCLVKDYFPEPVTVSWNSGALTSGVHTFPAVLQSSGLYSLSSVVTVPSSNFGTQTYTCNVDHKPSNTKVDKTVERKCCVECPPCPAPPVAGPSVFLFPPKPKDTLMISRTPEVTCVVVDVSHEDPEVQFNWYVDGVEVHNAKTKPREEQFNSTFRVVSVLTVVHQDWLNGKEYKCKVSNKGLPAPIEKTISKTKGQPREPQVYTLPPSREEMTKNQVSLTCLVKGFYPSDIAVEWESNGQPENNYKTTPPMLDSDGSFFLYSKLTVDKSRWQQGNVFSCSVMHEALHNHYTQKSLSLSPGK

SEQ ID NO: 69 - protein, 233 aa, Homo sapiens
MGSTAILGLLLAVLQGGRASYVLTQPPSVSVAPGQTARITCGGNNLGSKSVHWYQQKPGQAPVLVVYDDSDRPSWIPERFSGSNSGNTATLTISRGEAGDEADYYCQVWDSSSDHVVFGGGTKLTVLGQPKAAPSVTLFPPSSEELQANKATLVCLISDFYPGAVTVAWKADSSPVKAGVETTTPSKQSNNKYAASSYLSLTPEQWKSHRSYSCQVTHEGSTVEKTVAPTECS

SEQ ID NO: 70 - protein, 467 aa, Homo sapiens
MGSTAILGLLLAVLQGGRAQMQLVESGGGVVQPGRSLRLSCAASGFTFRTYGMHWVRQAPGKGLEWVAVIWYDGSNKHYADSVKGRFTITRDNSKNTLNLQMNSLRAEDTAVYYCARAPQWELVHEAFDIWGQGTMVTVSSASTKGPSVFPLAPCSRSTSESTAALGCLVKDYFPEPVTVSWNSGALTSGVHTFPAVLQSSGLYSLSSVVTVPSSNFGTQTYTCNVDHKPSNTKVDKTVERKCCVECPPCPAPPVAGPSVFLFPPKPKDTLMISRTPEVTCVVVDVSHEDPEVQFNWYVDGVEVHNAKTKPREEQFNSTFRVVSVLTVVHQDWLNGKEYKCKVSNKGLPAPIEKTISKTKGQPREPQVYTLPPSREEMTKNQVSLTCLVKGFYPSDIAVEWESNGQPENNYKTTPPMLDSDGSFFLYSKLTVDKSRWQQGNVFSCSVMHEALHNHYTQKSLSLSPGK

SEQ ID NO: 71 - protein, 234 aa, Homo sapiens
MGVPTHLLGLLLLWITHAICDIRMTQSPASLSASLGETVNIECLASEDIYSDLAWYQQKPGKSPQLLIYNANSLQNGVPSRFSGSGSGTQYSLKINSLQSEDVATYFCQQYNNYPPTFGGGTKLELKRADAAPTVSIFPPSTEQLATGGASVVCLMNNFYPRDISVKWKIDGTERRDGVLDSVTDQDSKDSTYSMSSTLSLTKADYESHNLYTCEVVHKTSSSPVVKSFNRNEC

SEQ ID NO: 72 - protein, 465 aa, Homo sapiens
MDIRLSLAFLVLFIKGVQCEVQLVESGGGLVQPANSLKLSCAASGFTFSDYAMAWVRQSPKKGLEWVATIIYDGSSTYYRDSVKGRFTISRDNAKSTLYLQMDSLRSEDTATYYCATGLGIATDYFDYWGQGVLVTVSSAETTAPSVYPLAPGTALKSNSMVTLGCLVKGYFPEPVTVTWNSGALSSGVHTFPAVLQSGLYTLTSSVTVPSSTWPSQTVTCNVAHPASSTKVDKKIVPRNCGGDCKPCICTGSEVSSVFIFPPKPKDVLTITLTPKVTCVVVDISQDDPEVHFSWFVDDVEVHTAQTRPPEEQFNSTFRSVSELPILHQDWLNGRTFRCKVTSAAFPSPIEKTISKPEGRTQVPHVYTMSPTKEEMTQNEVSITCMVKGFYPPDIYVEWQMNGQPQENYKNTPPTMDTDGSYFLYSKLNVKKEKWQQGNTFTCSVLHEGLHNHHTEKSLSHSPGK

SEQ ID NO: 73 - protein, 237 aa, Homo sapiens
MDMRVPAQLLGLLLLWLRGARCESALTQPASVSGSPGQSITISCTGTSSDVGGYNSVSWYQQHPGKAPKLMIYEVSNRPSGVSNRFSGSKSGNTASLTISGLQAEDEADYYCNSYTSTSMVFGGGTKLTVLGQPKAAPSVTLFPPSSEELQANKATLVCLISDFYPGAVTVAWKADSSPVKAGVETTTPSKQSNNKYAASSYLSLTPEQWKSHRSYSCQVTHEGSTVEKTVAPTECS

SEQ ID NO: 74 - protein, 460 aa, Homo sapiens
MDWTWRILFLVAAATGVHSEVQLVQSGAEVKKPGASVKVSCKASGYTLTSYGISWVRQAPGQGLEWMGWVSFYNGNTNYAQKLQGRGTMTTDPSTSTAYMELRSLRSDDTAVYYCARGYGMDVWGQGTTVTVSSASTKGPSVFPLAPCSRSTSESTAALGCLVKDYFPEPVTVSWNSGALTSGVHTFPAVLQSSGLYSLSSVVTVPSSNFGTQTYTCNVDHKPSNTKVDKTVERKCCVECPPCPAPPVAGPSVFLFPPKPKDTLMISRTPEVTCVVVDVSHEDPEVQFNWYVDGVEVHNAKTKPREEQFNSTFRVVSVLTVVHQDWLNGKEYKCKVSNKGLPAPIEKTISKTKGQPREPQVYTLPPSREEMTKNQVSLTCLVKGFYPSDIAVEWESNGQPENNYKTTPPMLDSDGSFFLYSKLTVDKSRWQQGNVFSCSVMHEALHNHYTQKSLSLSPGK

SEQ ID NO: 75 - protein, 234 aa, Homo sapiens
METPAQLLFLLLLWLPDTTGEIVMTQSPATLSVSPGERATLSCRASQSVSSNLAWYQQKPGQAPRLLIYGAATRATGIPARVSGSGSGTEFTLTISSLQSEDFAVYYCQQYNNWPLTFGGGTKVEIKRTVAAPSVFIFPPSDEQLKSGTASVVCLLNNFYPREAKVQWKVDNALQSGNSQESVTEQDSKDSTYSLSSTLTLSKADYEKHKVYACEVTHQGLSSPVTKSFNRGEC

SEQ ID NO: 76 - protein, 472 aa, Homo sapiens
MDMRVPAQLLGLLLLWLRGARCQVQLVESGGGVVQPGRSLRLSCAASGFTFSNYGMHWVRQAPGEGLEWVAAIWFDASDKYYADAVKGRFTISRDNSKNTLYLQMNSLRAEDTAVYYCARDQAIFGVVPDYWGQGTLVTVSSASTKGPSVFPLAPSSKSTSGGTAALGCLVKDYFPEPVTVSWNSGALTSGVHTFPAVLQSSGLYSLSSVVTVPSSSLGTQTYICNVNHKPSNTKVDKKVEPKSCDKTHTCPPCPAPELLGGPSVFLFPPKPKDTLMISRTPEVTCVVVDVSHEDPEVKFNWYVDGVEVHNAKTKPCEEQYGSTYRCVSVLTVLHQDWLNGKEYKCKVSNKALPAPIEKTISKAKGQPREPQVYTLPPSREEMTKNQVSLTCLVKGFYPSDIAVEWESNGQPENNYKTTPPVLDSDGSFFLYSKLTVDKSRWQQGNVFSCSVMHEALHNHYTQKSLSLSPGK

SEQ ID NO: 77 - protein, 231 aa, Homo sapiens
MAWIPLFLGVLAYCTGSVASYEVTQAPSVSVSPGQTASITCSGDKLGDKYACWYQQKPGQSPVLVIYQDSKRPSGIPERFSGSNSGNTATLTISGTQAMDEADYYCQAWDSSTAVFGGGTKLTVLGQPKAAPSVTLFPPSSEELQANKATLVCLISDFYPGAVTVAWKADSSPVKAGVETTTPSKQSNNKYAASSYLSLTPEQWKSHRSYSCQVTHEGSTVEKTVAPTECS

SEQ ID NO: 78 - protein, 467 aa, Homo sapiens
MDWTWSILFLVAAATGAHSQVQLVQSGAEVKKPGASVKVSCKASGYTFTSYGLSWVRQAPGQGLEWMGWIIPYNGNTNSAQKLQGRVTMTTDTSTSTAYMELRSLRSDDTAVYFCARDRDYGVNYDAFDIWGQGTMVTVSSASTKGPSVFPLAPCSRSTSESTAALGCLVKDYFPEPVTVSWNSGALTSGVHTFPAVLQSSGLYSLSSVVTVPSSNFGTQTYTCNVDHKPSNTKVDKTVERKCCVECPPCPAPPVAGPSVFLFPPKPKDTLMISRTPEVTCVVVDVSHEDPEVQFNWYVDGVEVHNAKTKPREEQFNSTFRVVSVLTVVHQDWLNGKEYKCKVSNKGLPAPIEKTISKTKGQPREPQVYTLPPSREEMTKNQVSLTCLVKGFYPSDIAVEWESNGQPENNYKTTPPMLDSDGSFFLYSKLTVDKSRWQQGNVFSCSVMHEALHNHYTQKSLSLSPGK

SEQ ID NO: 79 - protein, 235 aa, Homo sapiens
MAWAPLLLTLLAHCTGSWANFMLTQPHSVSESPGKTVAISCTRNSGSIASNSVQWYQQRPGSSPTTVIFEDNQRPSGVPDRFSGSIDSSSNSASLTISGLKTEDEADYYCQSYDSNNWVFGGGTKLTVLGQPKANPTVTLFPPSSEELQANKATLVCLISDFYPGAVTVAWKADGSPVKAGVETTKPSKQSNNKYAASSYLSLTPEQWKSHRSYSCQVTHEGSTVEKTVAPTECS

SEQ ID NO: 80 - protein, 470 aa, Homo sapiens
MEFGLSWVFLVALLRGVQCQVQLVESGGGVVQPGRSLRLSCAASGFTFSSYVMHWVRQAPGKGLEWVAVIWYDGSNKYYADSVKGRFTISRDNSKNTLYLQMNSLRAEDTAVYYCAREGYDYGEDYYYYGMDVWGQGTTVTVSSASTKGPSVFPLAPCSRSTSESTAALGCLVKDYFPEPVTVSWNSGALTSGVHTFPAVLQSSGLYSLSSVVTVPSSNFGTQTYTCNVDHKPSNTKVDKTVERKCCVECPPCPAPPVAGPSVFLFPPKPKDTLMISRTPEVTCVVVDVSHEDPEVQFNWYVDGVEVHNAKTKPREEQFNSTFRVVSVLTVVHQDWLNGKEYKCKVSNKGLPAPIEKTISKTKGQPREPQVYTLPPSREEMTKNQVSLTCLVKGFYPSDIAVEWESNGQPENNYKTTPPMLDSDGSFFLYSKLTVDKSRWQQGNVFSCSVMHEALHNHYTQKSLSLSPGK

SEQ ID NO: 81 - protein, 236 aa, Homo sapiens
MDMRVPAQLLGLLLLWLRGARCDIQMTQSPSSLSASVGDRVTITCRASQDISNYLNWYQQKPGKAPKLLIYYTSRLLSGVPSRFSGSGSGTDFTLTISSLQPEDFATYYCQQGDTLPYTFGGGTKVEIKRTVAAPSVFIFPPSDEQLKSGTASVVCLLNNFYPREAKVQWKVDNALQSGNSQESVTEQDSKDSTYSLSSTLTLSKADYEKHKVYACEVTHQGLSSPVTKSFNRGEC

SEQ ID NO: 82 - protein, 468 aa, Homo sapiens
MDWTWRILFLVAAATGAHSEVQLVQSGAEVKKPGASVKVSCKASGYTFTDYNMHWVRQAPGQGLEWMGEINPNSGGAGYNQKFKGRVTMTTDTSTSTAYMELRSLRSDDTAVYYCARLGYDDIYDDWYFDVWGQGTTVTVSSASTKGPSVFPLAPCSRSTSESTAALGCLVKDYFPEPVTVSWNSGALTSGVHTFPAVLQSSGLYSLSSVVTVPSSNFGTQTYTCNVDHKPSNTKVDKTVERKCCVECPPCPAPPVAGPSVFLFPPKPKDTLMISRTPEVTCVVVDVSHEDPEVQFNWYVDGVEVHNAKTKPREEQFNSTFRVVSVLTVVHQDWLNGKEYKCKVSNKGLPAPIEKTISKTKGQPREPQVYTLPPSREEMTKNQVSLTCLVKGFYPSDIAVEWESNGQPENNYKTTPPMLDSDGSFFLYSKLTVDKSRWQQGNVFSCSVMHEALHNHYTQKSLSLSPGK

SEQ ID NO: 83 - protein, 240 aa, Homo sapiens
MVLQTQVFISLLLWISGAYGDIVMTQSPDSLAVSLGERATINCKSSQSVLDSSDNKNYLAWYQQKPGQPPKLLIYWASNRESGVPDRFSGSGSGTDFTLTISSLQAEDVAVYYCQQYYSDPFTFGPGTKVDIKRTVAAPSVFIFPPSDEQLKSGTASVVCLLNNFYPREAKVQWKVDNALQSGNSQESVTEQDSKDSTYSLSSTLTLSKADYEKHKVYACEVTHQGLSSPVTKSFNRGEC

SEQ ID NO: 84 - protein, 465 aa, Homo sapiens
MDWTWSILFLVAAPTGAHSQVQLVQSGAEVKKPGASVKVSCKASGYTFTSYGISWVRQAPGQGLEWMGWISAYNGNTNYAQKLQGRVTMTTDTSTSTAYMELRSLRSDDTAVYYCARESWFGEVFFDYWGQGTLVTVSSASTKGPSVFPLAPCSRSTSESTAALGCLVKDYFPEPVTVSWNSGALTSGVHTFPAVLQSSGLYSLSSVVTVPSSNFGTQTYTCNVDHKPSNTKVDKTVERKCCVECPPCPAPPVAGPSVFLFPPKPKDTLMISRTPEVTCVVVDVSHEDPEVQFNWYVDGVEVHNAKTKPREEQFNSTFRVVSVLTVVHQDWLNGKEYKCKVSNKGLPAPIEKTISKTKGQPREPQVYTLPPSREEMTKNQVSLTCLVKGFYPSDIAVEWESNGQPENNYKTTPPMLDSDGSFFLYSKLTVDKSRWQQGNVFSCSVMHEALHNHYTQKSLSLSPGK

SEQ ID NO: 85 - protein, 236 aa, Homo sapiens
MDMRVPAQLLGLLLLWLRGARCDIQMTQSPSSVSASVGDRVTITCRASQGISSWLAWYQQKPGKAPKLLIYGASNLESGVPSRFSGSGSGTDFTLTISSLQPEDFANYYCQQANSFPWTFGQGTKVEIKRTVAAPSVFIFPPSDEQLKSGTASVVCLLNNFYPREAKVQWKVDNALQSGNSQESVTEQDSKDSTYSLSSTLTLSKADYEKHKVYACEVTHQGLSSPVTKSFNRGEC

SEQ ID NO: 86 - protein, 466 aa, Homo sapiens
MDMRVPAQLLGLLLLWLRGARCQVQLVQSGAEVKKPGASVKVSCKVSGYTLSDLSIHWVRQAPGKGLEWMGGFDPQDGETIYAQKFQGRVTMTEDTSTDTAYMELSSLKSEDTAVYYCATGSSSSWFDPWGQGTLVTVSSASTKGPSVFPLAPCSRSTSESTAALGCLVKDYFPEPVTVSWNSGALTSGVHTFPAVLQSSGLYSLSSVVTVPSSNFGTQTYTCNVDHKPSNTKVDKTVERKCCVECPPCPAPPVAGPSVFLFPPKPKDTLMISRTPEVTCVVVDVSHEDPEVQFNWYVDGVEVHNAKTKPREEQFNSTFRVVSVLTVVHQDWLNGKEYKCKVSNKGLPAPIEKTISKTKGQPREPQVYTLPPSREEMTKNQVSLTCLVKGFYPSDIAVEWESNGQPENNYKTTPPMLDSDGSFFLYSKLTVDKSRWQQGNVFSCSVMHEALHNHYTQKSLSLSPGK

SEQ ID NO: 87 - protein, 236 aa, Artificial sequence
  PD-1 antibody light chain
MDMRVPAQLLGLLLLWLRGARCDIQMTQSPSSVSASVGDRVTITCRASQGISNWLAWYQQKPGKAPKLLIFAASSLQSGVPSRFSGSGSGTDFTLTISSLQPEDFATYYCQQAESFPHTFGGGTKVEIKRTVAAPSVFIFPPSDEQLKSGTASVVCLLNNFYPREAKVQWKVDNALQSGNSQESVTEQDSKDSTYSLSSTLTLSKADYEKHKVYACEVTHQGLSSPVTKSFNRGEC

SEQ ID NO: 88 - protein, 472 aa, Artificial sequence
  PD-1 antibody heavy chain
MDMRVPAQLLGLLLLWLRGARCEVQLLESGGGLVQPGGSLRLSCAASGFTFSSYDMSWVRQAPGKGLEWVSLISGGGSQTYYAESVKGRFTISRDNSKNTLYLQMNSLRAEDTAVYFCASPSGHYFYAMDVWGQGTTVTVSSASTKGPSVFPLAPSSKSTSGGTAALGCLVKDYFPEPVTVSWNSGALTSGVHTFPAVLQSSGLYSLSSVVTVPSSSLGTQTYICNVNHKPSNTKVDKKVEPKSCDKTHTCPPCPAPELLGGPSVFLFPPKPKDTLMISRTPEVTCVVVDVSHEDPEVKFNWYVDGVEVHNAKTKPCEEQYGSTYRCVSVLTVLHQDWLNGKEYKCKVSNKALPAPIEKTISKAKGQPREPQVYTLPPSREEMTKNQVSLTCLVKGFYPSDIAVEWESNGQPENNYKTTPPVLDSDGSFFLYSKLTVDKSRWQQGNVFSCSVMHEALHNHYTQKSLSLSPGK